European Patent Application EP 4 650 363 A1, published November 19, 2025. Title: Rescue of chromosome cohesion in aged mammalian oocytes and eggs. Applicant: Max-Planck-Gesellschaft zur Förderung der Wissenschaften e.V. Application EP. The sequence listing filed with the application follows.

SEQUENCE LISTING (32 sequences)

SEQ ID NO: 1 - protein, 526 aa, Homo sapiens
AKERCLKKSFQDSLEDIKKRMKEKRNKNLAEIGKRRSFIAAPCQIITNTSTLLKNYQDNNKMLVLALENEKSKVKEAQDIILQLRKECYYLTCQLYALKGKLTSQQTVEPAQNQEICSSGMDPNSDDSSRNLFVKDLPQIPLEETELPGQGESFQIEDQIPTIPQDTLGVDFDSGEAKSTDNVLPRTVSVRSSLKKHCNSICQFDSLDDFETSHLAGKSFEFERVGFLDPLVNMHIPENVQHNACQWSKDQVNLSPKLIQPGTFTKTKEDILESKSEQTKSKQRDTQERKREEKRKANRRKSKRMSKYKENKSENKKTVPQKKMHKSVSSNDAYNFNLEEGVHLTPFRQKVSNDSNREENNESEVSLCESSGSGDDSDDLYLPTCKYIQNPTSNSDRPVTRPLAKRALKYTDEKETEGSKPTKTPTTTPPETQQSPHLSLKDITNVSLYPVVKIRRLSLSPKKNKASPAVALPKRRCTASVNYKEPTLASKLRRGDPFTDLCFLNSPIFKQKKDLRRSKKSMKQIQ

SEQ ID NO: 2 - protein, 1265 aa, Homo sapiens
MECPVMETGSLFTSGIKRHLKDKRISKTTKLNVSLASKIKTKILNNSSIFKISLKHNNRALAQALSREKENSRRITTEKMLLQKEVEKLNFENTFLRLKLNNLNKKLIDIEALMNNNLITAIEMSSLSEFHQSSFLLSASKKKRISKQCKLMRLPFARVPLTSNDDEDEDKEKMQCDNNIKSKTLPDIPSSGSTTQPLSTQDNSEVLFLKENNQNVYGLDDSEHISSIVDVPPRESHSHSDQSSKTSLMSEMRNAQSIGRRWEKPSPSNVTERKKRGSSWESNNLSADTPCATVLDKQHISSPELNCNNEINGHTNETNTEMQRNKQDLPGLSSESAREPNAECMNQIEDNDDFQLQKTVYDADMDLTASEVSKIVTVSTGIKKKSNKKTNEHGMKTFRKVKDSSSEKKRERSKRQFKNSSDVDIGEKIENRTERSDVLDGKRGAEDPGFIFNNEQLAQMNEQLAQVNELKKMTLQTGFEQGDRENVLCNKKEKRITNEQEETYSLSQSSGKFHQESKFDKGQNSLTCNKSKASRQTFVIHKLEKDNLLPNQKDKVTIYENLDVTNEFHTANLSTKDNGNLCDYGTHNILDLKKYVTDIQPSEQNESNINKLRKKVNRKTEIISGMNHMYEDNDKDVVHGLKKGNFFFKTQEDKEPISENIEVSKELQIPALSTRDNENQCDYRTQNVLGLQKQITNMYPVQQNESKVNKKLRQKVNRKTEIISEVNHLDNDKSIEYTVKSHSLFLTQKDKEIIPGNLEDPSEFETPALSTKDSGNLYDSEIQNVLGVKHGHDMQPACQNDSKIGKKPRLNVCQKSEIIPETNQIYENDNKGVHDLEKDNFFSLTPKDKETISENLQVTNEFQTVDLLIKDNGNLCDYDTQNILELKKYVTDRKSAEQNESKINKLRNKVNWKTEIISEMNQIYEDNDKDAHVQESYTKDLDFKVNKSKQKLECQDIINKHYMEVNSNEKESCDQILDSYKVVKKRKKESSCKAKNILTKAKNKLASQLTESSQTSISLESDLKHITSEADSDPGNPVELCKTQKQSTTTLNKKDLPFVEEIKEGECQVKKVNKMTSKSKKRKTSIDPSPESHEVMERILDSVQGKSTVSEQADKENNLENEKMVKNKPDFYTKAFRSLSEIHSPNIQDSSFDSVREGLVPLSVSSGKNVIIKENFALECSPAFQVSDDEHEKMNKMKFKVNRRTQKSGIGDRPLQDLSNTSFVSNNTAESENKSEDLSSERTSRRRRCTPFYFKEPSLRDKMRR

SEQ ID NO: 3 - RNA, 171 nt, Homo sapiens
  source 1..171: mol_type = transcribed RNA
cattctcagaaacttctttgtgatgtgtccattcaactcacagagttgaacctttcttttgatagagcagttttgaaacactctttttgtagaatctgcaagtggatatttggagcgctttgaggcctatggtggaaaaggaaatatcttcacataaaaactagacagaag

SEQ ID NO: 4 - protein, 517 aa, Mus musculus
MAKERCQKRSFQDTLEDIKNRMKEKRNKNLAGIGKRKSFIVAPGQVPTNTATLLRYYQDNNRLLVLALENEKSKVREAQDVILQLRKECYYLTCQLYALKEKLTSRQSEETTQNWKGRPSDVVSSIDNTTRDLSGKSLQQIAVEETDCPYQTTEPSPAVTPETQGCDFDSGKVESTDEVLPRTISIRRHLRKDFSNISHSTTLEDCKASPRVAQSLEVKGSRCREVTVTLHRLENVCLWNKDQISLCSRLINPAKITETEVILSSKPEQIESKHKRARKRRAEQRRTKQRCKSKSSLRSKGNKNKDKQGLPPTTLDGGIGSCDAYDFNLKGTVHPTPFRQKMNNGCNKETDSSNSEVSDLECSTSEDESDDLYLPPSKRLRDYRESERAVTRPRSKRGLQYPDGKERKEVLPSTAPTGIPPETQESPRCSLKDVTNILQCPRVKIRKPSLPPKRREDSPAVALTKRRCSTIKSYKEPTLASKLRRGDPFTDLCFLNSPIFKQKRGMRCPKRRTKQTQ

SEQ ID NO: 5 - protein, 1164 aa, Mus musculus
MEYPGIKVDTVTSGIQRRVKGRIAKTNLNVSLASKIKAKILNNSSIFKISLKHNNRALARALSKEKENSRRITTEKMQLQKEVEKLNFENTFLRLKLNTLNKKLVEIESHVSNDLLTAIEISSLSEFHQGSFLLSATKKQRNSKQCKPAHLPYARVLLTSENDDDDGADDKWQTKCNNRTISKTSPDSTSSVSRQPSSLHQCNLKAFPPKEDNQKTCGSGHLEHTSSVDILPNESHSDQSPKSSLSEMKTAPSPSLRREKLSHGNVTMRKKCVSSTPDILYVTDLDHQPTSSPGSNWNNEIHGHTNETSNNTQRNAECFLDLPSESSSEPDAKRMELVQKNTDSFHFQKTVYDAADMELTATDIGKIVAVSKSKKNQNKKKADCRKETFRKVKGASSDKKRESSKRECKDGSEVGAEEEADAARAERGAGVLDGRGDSEEPNCISSTEQPSQVNTQKKRTLQNSSDQENIQNTKRRQTYTTDEQEETNPFSRHSVKFLQDGKFDLCQKTLHHNLSKPSRQTFVIRKSEKDNLFPNQEDKDTISENLEVTNEFHIDDLSIEANENVCDHETQTMLDLKKSVSAQQNQTKINKTKQKINRRTKIISVMSQVYEDNDKDIHVLEKDNFPFHTQANKETTSGNLESSKEFESPLLFTRDNGSLRDCKTQNVLDLHKQIPDLYPDRNESQISKIPRQKVNRKTEVISGVKCFSNDQGVHCSEKDKSLLLQKDKDFPGTLKDLSEFDTPAFCNKDSAKSCDYKSEMLLGLKKHDPNMQPACQDDSKAGKKLRQKVNRKTEIISKITQIHENDRGSTHDSLNKKLCQKVNISKIISQMNQIYETINEDGNGFKSSIKDCEDIKSCDFGEINSNKKENYDPIQDPCTLVKKTKRKGSCKAGSSLAGAKNRCGLQLTDSSQVQSVPLDSGLRHHPNEADSGPGEQTNLPKMQKQSAGRSLGDAFSVSLGKEGSRPAKAVSKMTPKSKKRKLPLGCSPETHGTVEITPNTDLAKAVDSQQTEKENYLEKEKIAKRKPDFCTKVLKPLSETCSSNIKNSSLDSMCKSSLPLSISSRKTLMLEESSSLESTCIFQVGDAAHEKITTGTRNPHHRTQKSTPGSRTSLVLVDTSSVSDTNPANPENESEGQSSHPMRRKRQCVPLNLTEPSLRSKMRR

SEQ ID NO: 6 - RNA, 234 nt, Mus musculus
  source 1..234: mol_type = transcribed RNA
ggacctggaatatggcgagaaaactgaaaatcacggaaaatgagaaatacacactttaggacgtgaaatatggcgaggaaaactgaaaaaggtggaaaatttagaaatgtccactgtaggacgtggaatatggcaagaaaactgaaaatcatggaaaatgagaaacatccacttgacgacttgaaaaatgacgaaatcactaaaaaacgtgaaaaatgagaaatgcacactgaa

SEQ ID NO: 7 - RNA, 115 nt, Mus musculus
  source 1..115: mol_type = transcribed RNA
ggaaaatgataaaaaccacactttagaacatattagatgagtgagttacactgaaaacacattcgttggaaaccggcattgtagacagtgtatatcatgagtatactagaaacat

SEQ ID NO: 8 - DNA, 1578 bp, Homo sapiens
  source 1..1578: mol_type = genomic DNA
gccaaggaaagatgcctgaaaaagtcctttcaagatagtcttgaagacataaagaagcgaatgaaagagaaaaggaataaaaacttggcagagattggcaaacgcaggtcttttatagctgcaccatgccaaataatcaccaacacttctacactgctgaaaaattaccaagacaacaacaaaatgttagttttagctttggaaaatgaaaaatccaaagtgaaagaagcccaagatatcatcctacagctgagaaaagaatgttactatctcacatgtcagctatatgcattgaaaggaaaacttacatcacaacaaacagtagaacctgcacaaaatcaagaaatatgttcctctggaatggaccccaatagtgatgacagctccagaaatttatttgtgaaggatttaccgcaaattcctcttgaagaaactgaacttccaggacaaggagaatcatttcaaatagaagatcagatacctactattcctcaagacacactgggagttgattttgattcaggtgaagctaagtctactgataatgtcttacctagaactgtatctgttcgtagcagtttaaagaaacattgtaacagtatatgtcagtttgatagcttggatgattttgaaaccagtcatttggcagggaagtcttttgaattcgaaagagttggatttttagacccactagtaaacatgcacatacctgaaaatgtacaacacaatgcttgtcaatggagcaaggaccaagttaacttatcaccaaagctgattcagccaggaacgtttactaaaacaaaagaagacattttagaatctaaatctgaacaaactaaaagtaagcaaagagatacacaagaaagaaaaagagaagagaaaagaaaagctaacaggagaaaatcaaaacgtatgtcaaaatataaagagaataaaagcgaaaataaaaaaactgttccccaaaaaaaaatgcacaaatctgtcagttccaatgatgcttacaattttaatttggaagagggtgttcatcttactcctttccgacaaaaagtgagcaatgactctaatagagaagaaaacaacgagtctgaagtgagcctctgtgaatcaagtggttcaggagatgattccgatgacctctatttgcccacttgcaagtacattcagaatcccacgagcaattcagatagaccagtcaccaggcctctagctaaaagagcactgaaatacacagatgaaaaagagacggagggttctaagccaacaaaaactcctaccactacaccacctgaaactcagcagtcacctcatcttagcctgaaggatatcaccaatgtctccttgtatcctgttgtgaaaatcagaagactttctctttctccaaaaaagaataaagcaagcccagcagtggctctgcctaaacgtaggtgcacagccagcgtgaactataaggagcccaccctcgcttcgaaactgagaagaggggacccttttacagatttgtgttttttgaattctcctattttcaagcagaaaaaggatttgagacgttctaaaaaaagtatgaaacaaatacaa

SEQ ID NO: 9 - DNA, 3798 bp, Homo sapiens
  source 1..3798: mol_type = genomic DNA
atggagtgcccagtgatggaaactggctcactttttacctcaggaattaagagacatttgaaagacaaaagaatttcaaagactactaagttgaatgtttctcttgcttcaaaaataaaaacaaaaatactaaataattcttctattttcaaaatatctttaaagcacaacaacagggcattagctcaggctcttagtagagaaaaagagaattctcgaagaattacaactgaaaagatgctattgcaaaaagaagtagagaaactgaattttgagaacacatttcttcgcctaaagctaaataacttgaataagaagcttatagacatagaagctctcatgaacaataacttgataactgcaattgaaatgagcagtctttctgagttccatcagagttcctttctactgtcagctagcaagaagaaacgaattagtaaacagtgcaagttgatgcgtcttccatttgcaagggttccattaacttcaaatgatgatgaagatgaagataaagagaaaatgcagtgtgacaacaatattaaatcaaagacattacctgatattccctcttcaggatcaacaacacaacctttatcaactcaggataattcggaagtgttatttcttaaagaaaataatcaaaatgtatatggtttagatgattcagaacatatttcttctatagttgatgtacctcccagagaaagccattcccactcagaccaaagttctaagacttctctaatgagtgagatgagaaacgcccagtctattggccgcagatgggagaaaccatctcctagtaatgtgactgaaaggaagaagcgtgggtcatcttgggaatcaaataatctttctgcagacactccctgtgcaacagttttagataaacaacacatttcaagtccagaattaaattgcaataatgagataaatggtcatactaatgaaacaaatactgaaatgcaaagaaataaacaggatcttcctggcttatcttctgagtctgccagagaacctaatgcagagtgcatgaatcaaattgaggataatgatgactttcaattgcagaaaactgtgtatgatgctgacatggatttaactgctagtgaagtcagcaaaattgtcacagtctcaacaggcattaaaaagaaaagtaataaaaaaacaaatgaacatggaatgaaaactttcagaaaagtgaaagattccagctctgaaaaaaagagagaaagatcaaagagacagtttaaaaatagttcagatgtcgatattggggaaaagattgaaaacaggacagaaagatctgatgtcctggatggcaaaaggggtgcagaagatcccggttttattttcaataatgaacagctggctcagatgaatgaacagctggctcaggtgaatgaactaaagaaaatgacccttcaaactggctttgaacaaggtgacagagaaaatgtactgtgtaataaaaaggagaaaagaataacaaatgagcaagaggaaacatactctttatcccaaagttcaggtaaatttcaccaggagagtaaatttgataagggtcagaattccctaacttgtaataaaagtaaagcttctagacagacatttgtgattcacaaattagaaaaagataacttactcccaaaccaaaaggataaagtaaccatttatgaaaacctagacgtcacaaatgaatttcacacagccaatctttccaccaaagataatggaaatttatgtgattatgggacccacaatatattggatttgaaaaagtatgtcactgatattcaaccctcagagcaaaatgaatcaaacattaataagcttagaaagaaagtaaaccggaagacagaaataatttctggaatgaaccacatgtatgaggataatgataaagatgtggtgcatggcctaaaaaaaggtaatttttttttcaaaacccaagaggataaagaacctatctctgaaaacatagaagtttccaaagagcttcaaatcccagctctttctactagagataatgaaaatcaatgtgactataggacccagaatgtgttgggtttgcaaaagcagatcaccaatatgtaccccgttcagcaaaatgaatcaaaagttaataagaagcttaggcagaaagtaaatcggaagacagaaataatttctgaagtgaatcatttagataatgacaaaagtatagaatacacagttaaaagtcactcactctttttaacgcaaaaagataaggaaatcatccctggaaacctagaagacccaagtgagtttgaaacacctgctctttctaccaaagatagtggaaacctgtatgattctgagattcaaaatgttttgggggtgaaacatggccatgatatgcaacctgcttgtcaaaatgattcaaaaataggtaagaagcctagactaaatgtatgtcaaaagtcagaaataattcctgaaaccaaccaaatatatgagaatgataacaaaggtgtacatgacctagaaaaagataacttcttctctctaaccccaaaggataaagaaacaatttctgaaaatctacaagtcacaaatgaatttcaaacagttgatcttctcatcaaagataatggaaatttatgtgattatgacacccagaatatattggagttgaaaaagtatgttactgataggaaatctgctgagcaaaatgaatcaaaaataaataagctcaggaataaagtgaattggaagacagaaataatttctgaaatgaaccagatatatgaggataatgataaagatgcacatgtccaagaaagctatacaaaagatcttgattttaaagtaaataaatctaaacaaaaacttgaatgccaagacattatcaataaacactatatggaagtcaacagtaatgaaaaggaaagttgtgatcaaattttagattcctacaaagtagttaaaaaacgtaagaaagaatcatcatgcaaggcaaagaacattttgacaaaagctaagaacaaacttgcttcacagttaacagaatcttcacagacatctatctccttagaatctgatttaaaacatattactagtgaagcagattctgatccaggaaacccagttgaactatgtaagactcagaagcaaagcactaccactttgaataaaaaagatctcccttttgtggaagaaataaaagaaggagagtgtcaggttaaaaaggtaaataaaatgacatctaagtcaaagaaaaggaagacctccatagatccttctccagagagccatgaagtaatggaaagaatacttgacagcgttcagggaaagtctactgtatctgaacaagctgataaggaaaacaatttggagaatgagaaaatggtcaaaaataagccagacttttacacaaaggcatttagatctttgtctgagatacattcacctaacatacaagattcttcctttgacagtgttcgtgaaggtttagtacctttgagcgtttcttctggtaaaaatgtgataataaaagaaaattttgccttggagtgctccccagcctttcaagtaagtgatgatgagcatgagaagatgaacaagatgaaatttaaagtcaaccggagaacccaaaaatcaggaataggtgatagaccattacaggacttgtcaaataccagttttgtttcaaataacactgctgaatctgaaaataagtcagaagatctatcttcagaacggacaagcagaagaagaaggtgtactcctttctattttaaagagccaagcctcagagacaagatgagaagatga

SEQ ID NO: 10 - DNA, 1554 bp, Mus musculus
  source 1..1554: mol_type = genomic DNA
atggctaaggaaaggtgtcagaaaaggtcctttcaagatacccttgaagacattaagaatcgaatgaaagaaaaaaggaataaaaatttggcggggattgggaaacgcaagtcctttattgttgcaccgggccaagtacccactaacactgctacactactgagatattaccaagataacaacaggttgttagtcttggctttggaaaatgagaaatccaaagtgagagaagcacaggatgtcatcctgcaactgagaaaagaatgctactaccttacttgtcagctgtatgcattgaaagagaagctaacttcccgacaaagtgaagaaactactcagaactggaaaggacgtccctcagacgtggtctccagcattgacaatacgaccagggacttgtcagggaagtccttacagcaaattgctgttgaagaaactgattgtccttaccaaaccacagaaccaagtcctgctgttactccagagacacagggttgcgattttgattcaggtaaagttgagtctactgatgaagtcttacccagaactatatctatccgtcgccatttaaggaaagattttagtaatataagccactccacgactttggaggattgtaaagccagtccaagagtggcacagtctctggaagttaaaggaagtagatgtagagaagtaaccgtaaccctgcacagacttgaaaatgtttgtctgtggaacaaagaccaaattagcttatgttctagactgattaacccagcaaagattactgaaacagaagtcattttatcatctaaacctgaacaaatagaaagcaagcataaacgtgcacgaaaaagaagagcagagcaaagaagaaccaagcagagatgcaaatcaaaatcctcattgaggagtaaggggaacaaaaacaaagataagcagggtttaccccctactacactggatggaggtattggttcctgtgatgcttacgattttaatctaaaagggacggtccaccccacccctttccgacaaaaaatgaacaatggctgcaacaaagaaacggatagcagcaactcagaagtgagtgacctcgaatgcagtacctctgaggatgagtctgatgacctctacctgcctccctccaagcgcttgcgagactacagagagtcagagagagcagttaccaggcctcggtctaaaagaggacttcagtacccagatgggaaagagaggaaggaggtgctgccatctacagctcctactggtatcccacctgagactcaagagtcacctcgttgtagcctaaaggatgtcaccaatatcctgcagtgtcctagagtgaagatcaggaagccttctctgcctccaaagcggcgtgaagacagcccagcagtggctctgactaaacgcaggtgtagcaccatcaaaagctataaagagccaacactcgcttcaaagctaagaagaggggaccctttcacggacttgtgtttcttgaattctcctattttcaagcagaaaaggggtatgagatgtcctaaaagaagaaccaagcaaacacagtaa

SEQ ID NO: 11 - DNA, 3492 bp, Mus musculus
  source 1..3492: mol_type = genomic DNA
atggagtacccagggataaaagttgacactgttacctctggaattcagagacgagtgaagggcagaattgcaaagacaaatttgaatgtttctcttgcttcaaagatcaaagcaaaaatattaaacaattcttctattttcaagatctctctaaagcacaacaacagagcattagcgcgggcccttagtaaagagaaagagaattctcgaagaattactaccgaaaagatgcaattacagaaagaagtagagaaactgaattttgagaatacctttcttcgcttaaagttaaataccttgaataagaagcttgtagaaatagaatcgcatgtgagcaatgatttgttaactgcaattgaaataagcagtctttctgagttccaccaaggttcttttctcctgtcagctaccaagaaacaaaggaacagtaagcagtgcaagcctgcgcatcttccatatgcaagagttctgttaacttcagaaaatgatgatgatgatggtgctgatgataaatggcagacaaagtgtaacaacagaactatatcaaagacctcacctgatagtacctcttcagtatcaagacaaccttcatccttacatcagtgcaatttgaaagcattccctcctaaagaagataatcagaagacatgtgggtcaggtcatttagaacatacttcaagtgttgatatacttcctaatgagagccactcagatcaaagtcctaagagttctctgagtgagatgaaaactgctccatctcccagcctcagaagggaaaaattatcacatggtaatgtgactatgaggaagaagtgtgtgtcttcaactccagacattctgtatgtgacagatttagatcaccaaccaacttcaagtccaggatcaaattggaataatgagatacatggtcatactaatgaaaccagcaataacacgcaaagaaatgccgagtgttttcttgacttaccttctgagtcttccagtgagcctgacgcaaagcgcatggagctagtgcagaagaacaccgatagctttcacttccagaaaactgtatatgatgccgctgatatggagttaactgctactgacataggcaagattgtagcagtttcaaaaagcaagaaaaatcaaaataagaaaaaggcagactgtagaaaggagactttcagaaaagtgaaaggtgcaagctctgataaaaagagagaaagctcaaagagagaatgtaaagatggttcagaagtaggtgctgaggaagaggctgatgcagccagagcagaaagaggcgctggtgtcctggatggcagaggggattcagaagagccaaactgcatttccagtactgagcagccatctcaggtaaacacgcaaaagaaaagaaccctccagaacagctcagatcaggagaacattcaaaatacgaagaggaggcaaacatatacgacagatgagcaagaggaaacaaaccctttctccagacattcagtcaaatttcttcaagatggtaaatttgatctgtgtcagaaaaccctacatcataatttaagtaagccttctcgacagacatttgtgattcgtaagtcagaaaaagataacttatttccaaatcaagaagataaagacaccatttctgaaaacctagaagttacaaatgaatttcatatagatgatctttccatcgaagctaatgaaaatgtatgtgaccatgagactcagacaatgttggacttgaaaaagtctgtcagtgctcaacaaaatcaaacaaaaataaataagactaagcagaaaataaatcgaaggacaaaaataatttctgtcatgagccaagtatatgaggacaatgataaagatattcacgtcctagaaaaagacaactttccctttcatacccaagcaaataaagaaaccaccagtggaaacctagaaagttcaaaagaatttgaatcacctcttcttttcacaagagacaacggaagcttacgtgactgtaagacccagaatgttctggatctgcacaagcaaattcctgatctataccctgatcggaatgagtcccagattagcaaaatccctaggcaaaaagtaaatcgcaagacagaagtaatttctggagtgaaatgttttagtaatgaccaaggtgttcattgctcagaaaaggataagtctttgttactacaaaaggataaagacttcccaggaactttaaaagacttaagtgagtttgatacgcctgctttttgtaacaaagatagtgcaaagtcgtgtgattataagtctgaaatgctcttggggttgaaaaaacatgaccctaatatgcaacctgcttgtcaagatgattcaaaagcaggtaagaaacttagacaaaaggtaaatcgaaaaacagaaataatttctaaaatcacccaaatacatgaaaatgatagaggaagtacacatgactcattaaataagaagctctgtcagaaggttaatatatcaaaaatcatttctcaaatgaaccaaatatatgagactattaatgaagatggaaatggctttaaaagctctatcaaagattgcgaagatattaaaagttgtgactttggggaaatcaacagtaataaaaaggaaaattatgatccaattcaagatccttgcacactggttaaaaaaacaaagagaaagggatcatgtaaagcagggagcagtttggcaggagctaagaacaggtgtggtttgcagttaacagactcttcccaggtacagtctgtccccttagactctggcttaagacaccatccaaacgaagcagattctggtcctggagagcagactaacctgccaaagatgcagaaacaaagcgctgggaggtcactgggagatgctttctctgtgagtctgggaaaagaaggaagccgcccagccaaagcagttagtaaaatgacacccaaatcaaagaagagaaagctccctctcggttgttctcctgaaacccacgggacggtggagataacacccaacactgacctcgctaaggctgttgactcccaacagactgagaaggagaactatttggagaaggagaaaattgccaagaggaagccagatttttgtacaaaggtgttgaaacctttatctgagacatgttcatctaacataaagaattcttccttggacagtatgtgtaagagttcgctacctttgagtatttcttctagaaaaaccctgatgctggaagaaagttcttccctggagagtacatgcatctttcaagtaggtgatgccgctcatgagaagataacgacaggcacacgtaatccccaccacaggacacagaagtcgacaccgggtagcagaacgtccctggtcttggtggataccagttctgtttcagataccaaccctgctaaccccgagaatgagtcagaagggcagtcttcacacccaatgagaaggaaaagacagtgcgtccctctcaacctgacagagccaagccttagaagcaagatgaggaga

SEQ ID NO: 12 - DNA, 171 bp, Homo sapiens
  source 1..171: mol_type = genomic DNA
cattctcagaaacttctttgtgatgtgtccattcaactcacagagttgaacctttcttttgatagagcagttttgaaacactctttttgtagaatctgcaagtggatatttggagcgctttgaggcctatggtggaaaaggaaatatcttcacataaaaactagacagaag

SEQ ID NO: 13 - DNA, 234 bp, Mus musculus
  source 1..234: mol_type = genomic DNA
ggacctggaatatggcgagaaaactgaaaatcacggaaaatgagaaatacacactttaggacgtgaaatatggcgaggaaaactgaaaaaggtggaaaatttagaaatgtccactgtaggacgtggaatatggcaagaaaactgaaaatcatggaaaatgagaaacatccacttgacgacttgaaaaatgacgaaatcactaaaaaacgtgaaaaatgagaaatgcacactgaa

SEQ ID NO: 14 - DNA, 115 bp, Mus musculus
  source 1..115: mol_type = genomic DNA
ggaaaatgataaaaaccacactttagaacatattagatgagtgagttacactgaaaacacattcgttggaaaccggcattgtagacagtgtatatcatgagtatactagaaacat

SEQ ID NO: 15 - DNA, 28 bp, synthetic construct
  source 1..28: mol_type = other DNA
caccatggagtacccagggataaaagtt

SEQ ID NO: 16 - DNA, 21 bp, synthetic construct
  source 1..21: mol_type = other DNA
caccatgggacaaacaccaaa

SEQ ID NO: 17 - DNA, 27 bp, synthetic construct
  source 1..27: mol_type = other DNA
caccatggctaaggaaaggtgtcagaa

SEQ ID NO: 18 - DNA, 33 bp, synthetic construct
  source 1..33: mol_type = other DNA
ttactgtgtttgcttggttcttcttttaggaca

SEQ ID NO: 19 - DNA, 20 bp, synthetic construct
  source 1..20: mol_type = other DNA
gccaaggaaagatgcctgaa

SEQ ID NO: 20 - DNA, 23 bp, synthetic construct
  source 1..23: mol_type = other DNA
ttgtatttgtttcatactttttt

SEQ ID NO: 21 - DNA, 25 bp, synthetic construct
  source 1..25: mol_type = other DNA
aacctgatgttatcttggtaatatc

SEQ ID NO: 22 - DNA, 25 bp, synthetic construct
  source 1..25: mol_type = other DNA
aacctgatgttatcttggtaatatc

SEQ ID NO: 23 - DNA, 22 bp, synthetic construct
  source 1..22: mol_type = other DNA
ctaactcacattaattgcgttg

SEQ ID NO: 24 - DNA, 22 bp, synthetic construct
  source 1..22: mol_type = other DNA
attaatgtgagttagctcactc

SEQ ID NO: 25 - DNA, 21 bp, synthetic construct
  source 1..21: mol_type = other DNA
aacatgtgagcaaaaggccag

SEQ ID NO: 26 - DNA, 20 bp, synthetic construct
  source 1..20: mol_type = other DNA
cccagcttggagcgaacgac

SEQ ID NO: 27 - RNA, 21 nt, synthetic construct
  source 1..21: mol_type = other RNA
cagcaaattgctgttgaagaa

SEQ ID NO: 28 - RNA, 21 nt, synthetic construct
  source 1..21: mol_type = other RNA
caggagaattgcagagtacaa

SEQ ID NO: 29 - DNA, 20 bp, synthetic construct
  source 1..20: mol_type = other DNA
gcgaggaaaactgaaaaagg

SEQ ID NO: 30 - DNA, 18 bp, synthetic construct
  source 1..18: mol_type = other DNA
ttgccatattccacgtcc

SEQ ID NO: 31 - DNA, 17 bp, synthetic construct
  source 1..17: mol_type = other DNA
tcccgtttccaacgaat

SEQ ID NO: 32 - DNA, 17 bp, synthetic construct
  source 1..17: mol_type = other DNA
attcgttggaaacggga